European Patent Application EP 4 538 391 A1, published April 16, 2025. Title: Method for obtaining useful data for the prediction of fibrosis risk in a subject. Applicant: Baigene, S.L. The sequence listing filed with the application follows.

SEQUENCE LISTING (28 sequences)

SEQ ID NO: 1 - DNA, 30 bp, synthetic construct
  source 1..30: mol_type = other DNA; organism (original language) = constructo sintetico
ccatattctcctcttcctcctctatcttca

SEQ ID NO: 2 - DNA, 20 bp, synthetic construct
  source 1..20: mol_type = other DNA; organism (original language) = constructo sintetico
ctccagcaaccaggaatgtg

SEQ ID NO: 3 - DNA, 23 bp, synthetic construct
  source 1..23: mol_type = other DNA; organism (original language) = constructo sintetico
gggcagtggtactgaagaagaat

SEQ ID NO: 4 - DNA, 23 bp, synthetic construct
  source 1..23: mol_type = other DNA; organism (original language) = constructo sintetico
gggcagtggtactgaagaagaag

SEQ ID NO: 5 - DNA, 40 bp, synthetic construct
  source 1..40: mol_type = other DNA; organism (original language) = constructo sintetico
acttattctgttagaaatatctagaaaactactacgacct

SEQ ID NO: 6 - DNA, 20 bp, synthetic construct
  source 1..20: mol_type = other DNA; organism (original language) = constructo sintetico
acaacaggaccactgtcctt

SEQ ID NO: 7 - DNA, 30 bp, synthetic construct
  source 1..30: mol_type = other DNA; organism (original language) = constructo sintetico
tctcctaacaaactgtttcacatctttttt

SEQ ID NO: 8 - DNA, 30 bp, synthetic construct
  source 1..30: mol_type = other DNA; organism (original language) = constructo sintetico
tctcctaacaaactgtttcacatctttttc

SEQ ID NO: 9 - DNA, 38 bp, synthetic construct
  source 1..38: mol_type = other DNA; organism (original language) = constructo sintetico
aaatgataaatctataatgcattgtttctaaagccgat

SEQ ID NO: 10 - DNA, 21 bp, synthetic construct
  source 1..21: mol_type = other DNA; organism (original language) = constructo sintetico
tgttgatgcttcagagcatgg

SEQ ID NO: 11 - DNA, 29 bp, synthetic construct
  source 1..29: mol_type = other DNA; organism (original language) = constructo sintetico
catgggttcaagataagcatatctgtttc

SEQ ID NO: 12 - DNA, 29 bp, synthetic construct
  source 1..29: mol_type = other DNA; organism (original language) = constructo sintetico
catgggttcaagataagcatatctgtttg

SEQ ID NO: 13 - DNA, 21 bp, synthetic construct
  source 1..21: mol_type = other DNA; organism (original language) = constructo sintetico
ctgtgttctggctctccctgt

SEQ ID NO: 14 - DNA, 24 bp, synthetic construct
  source 1..24: mol_type = other DNA; organism (original language) = constructo sintetico
gccttgaagtaactgcacgaaatt

SEQ ID NO: 15 - DNA, 20 bp, synthetic construct
  source 1..20: mol_type = other DNA; organism (original language) = constructo sintetico
aggcagttctacaacagccc

SEQ ID NO: 16 - DNA, 20 bp, synthetic construct
  source 1..20: mol_type = other DNA; organism (original language) = constructo sintetico
aggcagttctacaacagccg

SEQ ID NO: 17 - DNA, 18 bp, synthetic construct
  source 1..18: mol_type = other DNA; organism (original language) = constructo sintetico
ccacctgctcccggaaga

SEQ ID NO: 18 - DNA, 22 bp, synthetic construct
  source 1..22: mol_type = other DNA; organism (original language) = constructo sintetico
cgtttcctctttaacctcagca

SEQ ID NO: 19 - DNA, 19 bp, synthetic construct
  source 1..19: mol_type = other DNA; organism (original language) = constructo sintetico
gcatccctgagaacgaggc

SEQ ID NO: 20 - DNA, 19 bp, synthetic construct
  source 1..19: mol_type = other DNA; organism (original language) = constructo sintetico
gcatccctgagaacgaggt

SEQ ID NO: 21 - DNA, 40 bp, synthetic construct
  source 1..40: mol_type = other DNA; organism (original language) = constructo sintetico
tgaatttcatccttaagttctttttatttaataaatgtta

SEQ ID NO: 22 - DNA, 28 bp, synthetic construct
  source 1..28: mol_type = other DNA; organism (original language) = constructo sintetico
gtgtatgtttgaaattttccctaacgaa

SEQ ID NO: 23 - DNA, 36 bp, synthetic construct
  source 1..36: mol_type = other DNA; organism (original language) = constructo sintetico
tttaaaatatttgggaaaaaactagcttataataac

SEQ ID NO: 24 - DNA, 36 bp, synthetic construct
  source 1..36: mol_type = other DNA; organism (original language) = constructo sintetico
tttaaaatatttgggaaaaaactagcttataataat

SEQ ID NO: 25 - DNA, 20 bp, synthetic construct
  source 1..20: mol_type = other DNA; organism (original language) = constructo sintetico
ggcccaacccagagccatta

SEQ ID NO: 26 - DNA, 27 bp, synthetic construct
  source 1..27: mol_type = other DNA; organism (original language) = constructo sintetico
cacaccgtttatttaaatgctttctca

SEQ ID NO: 27 - DNA, 22 bp, synthetic construct
  source 1..22: mol_type = other DNA; organism (original language) = constructo sintetico
ccagagccagtgttcttgttca

SEQ ID NO: 28 - DNA, 21 bp, synthetic construct
  source 1..21: mol_type = other DNA; organism (original language) = constructo sintetico
cagagccagtgttcttgttcg